European Patent Application EP 4 516 924 A1, published March 5, 2025. Title: 重组酶介导的全冻干恒温扩增体系及其制备方法和应用. Applicant: 圣湘生物科技股份有限公司. Application CN. The sequence listing filed with the application follows.

SEQUENCE LISTING (6 sequences)

SEQ ID NO: 1 - DNA, 32 bp, Artificial sequence
  source 1..32: mol_type = other DNA
ggtcgaaacgtacgttctctctatcattccat

SEQ ID NO: 2 - DNA, 30 bp, Artificial sequence
  source 1..30: mol_type = other DNA
cagtgagcgaggactgcagcgtagacggtt

SEQ ID NO: 3 - DNA, 46 bp, Artificial sequence
  source 1..46: mol_type = other DNA
tgcagggaagaacgcagatctcgaggctctcatggagtggataaag

SEQ ID NO: 4 - DNA, 34 bp, Artificial sequence
  source 1..34: mol_type = other DNA
caacaccctgacaaaatcaacaatatagtaacaa

SEQ ID NO: 5 - DNA, 33 bp, Artificial sequence
  source 1..33: mol_type = other DNA
gcaagtctgctggcacagatgactggaacatag

SEQ ID NO: 6 - DNA, 52 bp, Artificial sequence
  source 1..52: mol_type = other DNA
ttcagtacaatgttctagaaaaagatgatgatcctgcatcactaacaatatg